European Patent Application EP 4 628 501 A1, published October 8, 2025. Title: Conjugate comprising peptide of novel sequence and glycyrrhizin, and pharmaceutical composition for preventing or treating obesity comprising same. Applicant: IUCF-HYU. Application KR PCT/KR2023/019124, filed June 6, 2024. The sequence listing filed with the application follows.

SEQUENCE LISTING (22 sequences)

SEQ ID NO: 1 - protein, 9 aa, artificial sequence
GKGRRAKDC

SEQ ID NO: 2 - protein, 10 aa, artificial sequence
KGRRAEDGSV

SEQ ID NO: 3 - protein, 5 aa, artificial sequence
KGGRA

SEQ ID NO: 4 - protein, 5 aa, artificial sequence
KGRRA

SEQ ID NO: 5 - protein, 5 aa, artificial sequence
GGRAK

SEQ ID NO: 6 - protein, 5 aa, artificial sequence
GRRAK

SEQ ID NO: 7 - protein, 5 aa, artificial sequence
GRAKD

SEQ ID NO: 8 - protein, 5 aa, artificial sequence
RRAED

SEQ ID NO: 9 - protein, 5 aa, artificial sequence
RAEDG

SEQ ID NO: 10 - protein, 5 aa, artificial sequence
KDGSV

SEQ ID NO: 11 - protein, 7 aa, artificial sequence
KGGRAKR

SEQ ID NO: 12 - protein, 7 aa, artificial sequence
KGGRAKK

SEQ ID NO: 13 - protein, 7 aa, artificial sequence
KGGRAKH

SEQ ID NO: 14 - protein, 7 aa, artificial sequence
KGRRAKD

SEQ ID NO: 15 - protein, 7 aa, artificial sequence
KGRRAKR

SEQ ID NO: 16 - protein, 7 aa, artificial sequence
KGRRAKK

SEQ ID NO: 17 - protein, 7 aa, artificial sequence
KGRRAKH

SEQ ID NO: 18 - protein, 7 aa, artificial sequence
KGGRAED

SEQ ID NO: 19 - protein, 7 aa, artificial sequence
GRRAKDG

SEQ ID NO: 20 - protein, 7 aa, artificial sequence
RRAEGSV

SEQ ID NO: 21 - protein, 7 aa, artificial sequence
RAKDGSV

SEQ ID NO: 22 - protein, 7 aa, artificial sequence
KGGRAKD